European Patent Application EP 4 516 919 A1, published March 5, 2025. Title: 一种N-乙酰-D-氨基酸、D-氨基酸、D-氨基酸衍生物的制备方法. Applicant: 元素驱动（杭州）生物科技有限公司. The sequence listing filed with the application follows.

SEQUENCE LISTING (2 sequences)

SEQ ID NO: 1 - DNA, 1353 bp, Pseudomonas putida
  source 1..1353: mol_type = genomic DNA
atgggtaaattagacaaagcgtctaaattaattgatgaagaaaacaagtattatgcacgttcggcgcgcatcaattactacaatctggtaattgaccacgcacacggggcaaccttagtggatgtcgacggcaataaatacattgatttgctggcaagcgcatctgcaattaacgttggccacacccatgaaaaagtcgtcaaggcgatcgccgatcaagctcaaaaattaattcattacactcccgcttattttcaccatgttcctggaatggaactttccgaaaagttagcgaaaattgcgccgggaaattcaccgaaaatggttagtttcggtaactccggctcagacgcaaacgatgcaattatcaagtttgcgagagcctatactggccgtcaatacattgtttcctatatgggttcctatcatgggtcaacttatggttcgcaaaccttatcaggaagtagtcttaacatgacacgtaaaattgggccaatgcttccaagcgtggtgcacgttccgtatccagattcatatcgaacctatccgggagaaaccgagcacgacgtttcactaaggtattttaacgaattcaagaagccattcgaatcattcttacccgctgatgaaactgcgtgtgtcttgattgaaccaattcaaggcgatggcggcatcatcaaagcccctgaagaatatatgcagttagtttataaattctgtcatgaacacgggatcctgtttgcgattgatgaagtcaatcaaggactcggccggaccggtaagatgtgggcaatccaacaattcaaagacatcgaacctgatttaatgtctgtcggtaagtcgctggcgtctggaatgccccttagtgcagtgattggtaagaaagaggtcatgcagagtttggatgcacctgcgcacctgtttaccactgccggcaatccggtttgttccgcagcttcgctggctaccttggatgtgatcgaatatgaaggcttggttgaaaaatcggccaccgatggtgcatacgccaaacaacgtttcttagagatgcagcaacgccatcccatgattggtgatgtccgaatgtggggcctcaatggtggaatcgaattggtcaaggatcctaagaccaaggaacccgacagtgacgctgccaccaaagtgatctactatgcctttgcacacggcgtcgttatcatcactttggcaggcaatattctgcgtttccagccgccgttggtcattccaagagagcaactcgaccaagcgcttcaagtgcttgacgacgcgtttaccgcagttgaaaatggtgaggttaccattcccaaggatacaggtaaaattggctggtaa

SEQ ID NO: 2 - DNA, 540 bp, Saccharomyces cerevisiae
  source 1..540: mol_type = genomic DNA
atgaaaaagaccccagacccatctccaccttttgcaagcacgaagaacgtaggcatgtcaaacgaagaaccggaaaaaatggttaacgatcgaattgtggtgaaggccatcgagccaaaagatgaggaagcctggaacaaactgtggaaggagtatcagggtttccaaaaaacggttatgcctccggaagtagccaccactaccttcgcaaggtttatagaccctacggtcaaactatggggtgctctagcctttgacaccgagaccggcgatgcaattggctttgcacactacctgaaccatttgacgtcgtggcatgtcgaagaagttgtctacatgaatgacttatatgtcactgaacgcgcaagagtcaaaggcgtaggtagaaagctcatagaatttgtatacagccgtgccgatgagctcggtacgcctgcagtgtactgggttacagaccattacaatcaccgcgcacagttgctgtacaccaaagtggcttacaagacagataaggttctttacaagagaaacggatactaa